European Patent Application EP 4 321 625 A1, published February 14, 2024. Title: A method of predicting a prognosis and a response to anticancer therapy of cancer patients. Applicant: INDUSTRY FOUNDATION OF CHONNAM NATIONAL UNIVERSITY. The sequence listing filed with the application follows.

SEQUENCE LISTING (4 sequences)

SEQ ID NO: 1 - DNA, 37 bp, Artificial Sequence
  tel1
ggtttttgagggtgagggtgagggtgagggtgagggt

SEQ ID NO: 2 - DNA, 39 bp, Artificial Sequence
  tel2
tcccgactatccctatccctatccctatccctatcccta

SEQ ID NO: 3 - DNA, 23 bp, Artificial Sequence
  36B4u
cagcaagtgggaaggtgtaatcc

SEQ ID NO: 4 - DNA, 25 bp, Artificial Sequence
  36B4d
cccattctatcatcaacgggtacaa